European Patent Application EP 4 582 458 A1, published July 9, 2025. Title: MICELLE COMPRISING AMPHIPHILIC PEPTIDE, AND ANTIGEN CARRIER NANOPARTICLE USING SAME. Applicant: RtAb Co., Ltd. Application WO PCT/KR2023/012758, filed August 29, 2023. The sequence listing filed with the application follows.

SEQUENCE LISTING (11 sequences)

SEQ ID NO: 1 - protein, 9 aa, synthetic construct
RRRVVVVVV

SEQ ID NO: 2 - protein, 11 aa, synthetic construct
RRRRVVVVVVV

SEQ ID NO: 3 - protein, 9 aa, synthetic construct
EEEVVVVVV

SEQ ID NO: 4 - protein, 11 aa, synthetic construct
EEEEVVVVVVV

SEQ ID NO: 5 - protein, 10 aa, synthetic construct
SDLGQHTLIV

SEQ ID NO: 6 - protein, 8 aa, synthetic construct
LEDTLSSE

SEQ ID NO: 7 - protein, 11 aa, synthetic construct
PGSQRYSQTGN

SEQ ID NO: 8 - protein, 10 aa, synthetic construct
APTSEIQLTD

SEQ ID NO: 9 - protein, 10 aa, synthetic construct
SSITEAELTG

SEQ ID NO: 10 - protein, 10 aa, synthetic construct
ASTVEAILPE

SEQ ID NO: 11 - protein, 10 aa, synthetic construct
SPSVEVKLPD